European Patent Application EP 4 177 275 A1, published May 10, 2023. Title: COAGULATION FACTOR XI (FXI) BINDING PROTEIN. Applicant: Suzhou Alphamab Co., Ltd. The sequence listing filed with the application follows.

SEQUENCE LISTING (343 sequences)

SEQ ID NO: 1 - protein, 123 aa, Artificial sequence
  ARTIFICIAL SEQUENCE
QVQLQESGGGSVQAGGSLRLSCAASGYTYSFNSMGWFRQAPGKEREGVAVIYLGSTHYADSVKGRFTISQDNAKNMVYLQMNSLKPEDTAMYYCAADLLEYDGTWFGSTYNYWGQGTQVTVSS

SEQ ID NO: 2 - protein, 121 aa, Artificial sequence
  ARTIFICIAL SEQUENCE
QVQLQESGGGLVQPGGSLRLSCAASGLTFSLYDMSWVRQAPGKGLEGVSGINSGDGSTYYADSVKGRFTISRDNAKNTLYLQMNSLKTEDTAVYYCATGRTRETYFREDDWGQGTQVTVSS

SEQ ID NO: 3 - protein, 120 aa, Artificial sequence
  ARTIFICIAL SEQUENCE
QVQLQESGGGLVQPGGSLRLSCAASGLRFSVYDMSWVRQAPGKGLEGVSGIDSGGGSTYYADSVKGRFTISRDDAKNTLYLQMNSLKTEDTAVYYCATGLGGSWYREPDWGQGTQVTVSS

SEQ ID NO: 4 - protein, 120 aa, Artificial sequence
  ARTIFICIAL SEQUENCE
QVQLQESGGGSVQAGGSLRLSCAGDGYTYSMGAMAWFRQAPGKEREGVALIATSSGFISYTDSVKGRFTISQDDAKIYLQMNSLKPEDTAMYYCAAGTQFSWSPGSYNYWGQGTQVTVSS

SEQ ID NO: 5 - protein, 121 aa, Artificial sequence
  ARTIFICIAL SEQUENCE
QVQLQESGGGLVQPGGSLRLSCAASGFTFSNYDMSWVRQAPGKGLEGVSGINSGGGHPHYADSVKGRFTISRDNAKNTLYLQMNSLKTEDTAVYFCATDEGERYGEDFGYWGQGTQVTVSS

SEQ ID NO: 6 - protein, 120 aa, Artificial sequence
  ARTIFICIAL SEQUENCE
QVQLQESGGGLVQPGGSLRVSCAASGFTFSLYDMSWVRQAPGKEREGVSGINSDDGSTSYADSVKGRFTISRDNAKNTLYLQMNSLKTEDTAVYYCATGVGARWFREDDWGQGTQVTVSS

SEQ ID NO: 7 - protein, 120 aa, Artificial sequence
  ARTIFICIAL SEQUENCE
QVQLQESGGGLVQPGGSLRLSCAASGLRFEIYDMSWVRQAPGKGLEGVSAINSGGGSTYYADSVKGRFTISRDDVKNTLYLQMNSLKTEDTAVYYCATGDGGSWYRDGDWGQGTQVTVSS

SEQ ID NO: 8 - protein, 121 aa, Artificial sequence
  ARTIFICIAL SEQUENCE
QVQLQESGGGLVQPGGSLRLSCVASGLTFSLYDMSWVRQAPGKGLEGVSGISGESGGSTYYADSVKGRFTISRDNAKNTLYLQMNSLKTEDTAVYYCATGDRGTWYREDDWGQGTQVTVSS

SEQ ID NO: 9 - protein, 120 aa, Artificial sequence
  ARTIFICIAL SEQUENCE
QVQLQESGGGLVQPGGSLRLSCAASGLRFSIYDMSWVRQAPGKGLEGVSGINSGGGSTYYADSVKGRFTISRDNAKNTLYLQMNSLKTEDTAVYYCATGLGGSWFREDDWGQGTQVTVSS

SEQ ID NO: 10 - protein, 117 aa, Artificial sequence
  ARTIFICIAL SEQUENCE
QVQLQESGGGSVQAGGSLGLSCTASGFTFDDSDMGWYRQAPGNECELVSTISSDGRGFYADSVKGRFTISQDRAKNTVYLHMNSLKPEDTAVYYCAAGWYGSFCSGLGQGTQVTVSS

SEQ ID NO: 11 - protein, 120 aa, Artificial sequence
  ARTIFICIAL SEQUENCE
QVQLQESGGGSVQAGGSLRLSCAASGLRFSIYDWSWVRQAPGKGLEWVSAINSGGGVTSYADSVKGRVTISRDNAKNTLYLQMHSLKTEDTAVYYCATGDGGSWYRDGDWGQGTQVTVSS

SEQ ID NO: 12 - protein, 136 aa, Artificial sequence
  ARTIFICIAL SEQUENCE
QVQLQESGGDSVQAGGSLRLSCAASGLISTGLISTRHCMSWFRQAPGKEREEVAVIGSDGSTRYGDFAKGRFTISKDTAKNTLYLQMNSLEPEDTAMYYCAAGPLVSTASRRRTRCPEGPRENIYWGQGTQVTVSS

SEQ ID NO: 13 - protein, 120 aa, Artificial sequence
  ARTIFICIAL SEQUENCE
QVQLQESGGGLVQPGGSLRLSCAASGFTFSLYDMSWVRQAPGQGLEWVSAITNPGGSTYYADSVKDRFTISRDNAKNTLYLQMNSLKTEDTAVYYCAIGRRATFQREKDWGQGTQVTVSS

SEQ ID NO: 14 - protein, 130 aa, Artificial sequence
  ARTIFICIAL SEQUENCE
QVQLQESGGGSVQAGGSLRLSCAASGHTYSSNYCMAWFRQAPGKEREGVAAIYSDGSTSYADSVKGRFTISKDNAKNTLYLQIDSLKPEDTSLYYCAATAYEGSWTGKQPLCLLYEYTYWGQGTQVTVSS

SEQ ID NO: 15 - protein, 119 aa, Artificial sequence
  ARTIFICIAL SEQUENCE
QVQLQESGGGLVQPGGSLRLSCAASGFTFSLYDMSWVRQAPGKGLDGVSGIGGDGGSTYYADSVKGRFAISRDDAKNTLYLQMNSLKIEDTAVYYCALGRPPYTDYDSRGQGTQVTVSS

SEQ ID NO: 16 - protein, 124 aa, Artificial sequence
  ARTIFICIAL SEQUENCE
QVQLQESGGGSVQAGGSLRLSCAASGFTASSNFMGWFRQAPGKEREGVAAIYTGGASTFYADSVKGRFTISQDNAKNTVYLEMDTLKPEDTAMYYCAAAPRWIAPLRADRYEYWGQGTQVTVSS

SEQ ID NO: 17 - protein, 126 aa, Artificial sequence
  ARTIFICIAL SEQUENCE
QVQLQESGGGSVQAGGSLRLSCTASEFTFDDSDMAWYRQAPGNECELVSTITSDGGTYYADSVKGRFTISQDNAKNTMYLQMNNLKPEDTAVYYCAADQWGSAEGDCTSSYPGGYWGQGTQVTVSS

SEQ ID NO: 18 - protein, 120 aa, Artificial sequence
  ARTIFICIAL SEQUENCE
QVQLQESGGGLVQPGGSLRLSCAASGFTFSLYDMSWVRQSPGKGLEGVSAIDSGDGRTYYADSVKGRFTISRDDAKNTLYLQMNSLKTGDTAVYYCANGGRGSWFRESDWGQGTQVTVSS

SEQ ID NO: 19 - protein, 119 aa, Artificial sequence
  ARTIFICIAL SEQUENCE
QVQLQESGGRLVQPGGSLRLSCVASGFTFEYYDMSWVRQAPGKGLEGVSAIDARSITDYADAVKGRFTISRDNAKNTLYLQLNNLKTEDTAMYYCANGGRIGWFREDDWGQGTQVTVSS

SEQ ID NO: 20 - protein, 124 aa, Artificial sequence
  ARTIFICIAL SEQUENCE
QVQLQESGGGSVQAGGSLRLSCVASGYTFNNNFVGWFRQAPGKEREGVAAIYSLGGSTYYADSVKGRFTISQDNAKNTVYLQMDSLKPEDTATYYCAGAITWVPPLSHRRYTYWGQGTQVTVSS

SEQ ID NO: 21 - protein, 124 aa, Artificial sequence
  ARTIFICIAL SEQUENCE
QVQLQESGGDSVQAGGSLRLSCIASGFTFDDSDMGWYRQAPGHQCEFVSHITNDGTTYYADSVKGRFTISRDNAKNTVYLQMNSLKPEDAAVYYCAADAWGGGRSTCVNPIGYWGQGTQVTVSS

SEQ ID NO: 22 - protein, 120 aa, Artificial sequence
  ARTIFICIAL SEQUENCE
QVQLQESGGGSVQAGGSLRLSCVASGFTGCRNIMSWYRQAPGKDREFVSAIDSDGVDYADSVKGRFSISQHNDKKTMYLQMTSLKLEDTAMYYCRRVDFGTTSQCRGNYWGQGTQVTVSS

SEQ ID NO: 23 - protein, 124 aa, Artificial sequence
  ARTIFICIAL SEQUENCE
QVQLQESGGGSVQAGGSLRLSCAASGYTFSNNFVGWFRQAPGKKREGVATIYTLGSSTYYADSVKGRFTISQDNAKNTLYLEMNSLKPEDTAMYYCAAARGWVSPLDPARFVYWGQGTQVTVSS

SEQ ID NO: 24 - protein, 5 aa, Artificial sequence
  ARTIFICIAL SEQUENCE
FNSMG

SEQ ID NO: 25 - protein, 14 aa, Artificial sequence
  ARTIFICIAL SEQUENCE
IYLGSTHYADSVKG

SEQ ID NO: 26 - protein, 16 aa, Artificial sequence
  ARTIFICIAL SEQUENCE
DLLEYDGTWFGSTYNY

SEQ ID NO: 27 - protein, 10 aa, Artificial sequence
  ARTIFICIAL SEQUENCE
GYTYSFNSMG

SEQ ID NO: 28 - protein, 7 aa, Artificial sequence
  ARTIFICIAL SEQUENCE
IYLGSTH

SEQ ID NO: 29 - protein, 16 aa, Artificial sequence
  ARTIFICIAL SEQUENCE
DLLEYDGTWFGSTYNY

SEQ ID NO: 30 - protein, 7 aa, Artificial sequence
  ARTIFICIAL SEQUENCE
GYTYSFN

SEQ ID NO: 31 - protein, 3 aa, Artificial sequence
  ARTIFICIAL SEQUENCE
LGS

SEQ ID NO: 32 - protein, 16 aa, Artificial sequence
  ARTIFICIAL SEQUENCE
DLLEYDGTWFGSTYNY

SEQ ID NO: 33 - protein, 8 aa, Artificial sequence
  ARTIFICIAL SEQUENCE
GYTYSFNS

SEQ ID NO: 34 - protein, 5 aa, Artificial sequence
  ARTIFICIAL SEQUENCE
YLGST

SEQ ID NO: 35 - protein, 18 aa, Artificial sequence
  ARTIFICIAL SEQUENCE
AADLLEYDGTWFGSTYNY

SEQ ID NO: 36 - protein, 5 aa, Artificial sequence
  ARTIFICIAL SEQUENCE
LYDMS

SEQ ID NO: 37 - protein, 17 aa, Artificial sequence
  ARTIFICIAL SEQUENCE
GINSGDGSTYYADSVKG

SEQ ID NO: 38 - protein, 12 aa, Artificial sequence
  ARTIFICIAL SEQUENCE
GRTRETYFREDD

SEQ ID NO: 39 - protein, 10 aa, Artificial sequence
  ARTIFICIAL SEQUENCE
GLTFSLYDMS

SEQ ID NO: 40 - protein, 10 aa, Artificial sequence
  ARTIFICIAL SEQUENCE
GINSGDGSTY

SEQ ID NO: 41 - protein, 12 aa, Artificial sequence
  ARTIFICIAL SEQUENCE
GRTRETYFREDD

SEQ ID NO: 42 - protein, 6 aa, Artificial sequence
  ARTIFICIAL SEQUENCE
NSGDGS

SEQ ID NO: 43 - protein, 6 aa, Artificial sequence
  ARTIFICIAL SEQUENCE
NSGDGS

SEQ ID NO: 44 - protein, 12 aa, Artificial sequence
  ARTIFICIAL SEQUENCE
GRTRETYFREDD

SEQ ID NO: 45 - protein, 8 aa, Artificial sequence
  ARTIFICIAL SEQUENCE
GLTFSLYD

SEQ ID NO: 46 - protein, 8 aa, Artificial sequence
  ARTIFICIAL SEQUENCE
INSGDGST

SEQ ID NO: 47 - protein, 14 aa, Artificial sequence
  ARTIFICIAL SEQUENCE
ATGRTRETYFREDD

SEQ ID NO: 48 - protein, 5 aa, Artificial sequence
  ARTIFICIAL SEQUENCE
VYDMS

SEQ ID NO: 49 - protein, 17 aa, Artificial sequence
  ARTIFICIAL SEQUENCE
GIDSGGGSTYYADSVKG

SEQ ID NO: 50 - protein, 11 aa, Artificial sequence
  ARTIFICIAL SEQUENCE
GLGGSWYREPD

SEQ ID NO: 51 - protein, 10 aa, Artificial sequence
  ARTIFICIAL SEQUENCE
GLRFSVYDMS

SEQ ID NO: 52 - protein, 10 aa, Artificial sequence
  ARTIFICIAL SEQUENCE
GIDSGGGSTY

SEQ ID NO: 53 - protein, 11 aa, Artificial sequence
  ARTIFICIAL SEQUENCE
GLGGSWYREPD

SEQ ID NO: 54 - protein, 7 aa, Artificial sequence
  ARTIFICIAL SEQUENCE
GLRFSVY

SEQ ID NO: 55 - protein, 6 aa, Artificial sequence
  ARTIFICIAL SEQUENCE
DSGGGS

SEQ ID NO: 56 - protein, 11 aa, Artificial sequence
  ARTIFICIAL SEQUENCE
GLGGSWYREPD

SEQ ID NO: 57 - protein, 8 aa, Artificial sequence
  ARTIFICIAL SEQUENCE
GLRFSVYD

SEQ ID NO: 58 - protein, 8 aa, Artificial sequence
  ARTIFICIAL SEQUENCE
IDSGGGST

SEQ ID NO: 59 - protein, 13 aa, Artificial sequence
  ARTIFICIAL SEQUENCE
ATGLGGSWYREPD

SEQ ID NO: 60 - protein, 5 aa, Artificial sequence
  ARTIFICIAL SEQUENCE
MGAMA

SEQ ID NO: 61 - protein, 17 aa, Artificial sequence
  ARTIFICIAL SEQUENCE
LIATSSGFISYTDSVKG

SEQ ID NO: 62 - protein, 13 aa, Artificial sequence
  ARTIFICIAL SEQUENCE
GTQFSWSPGSYNY

SEQ ID NO: 63 - protein, 10 aa, Artificial sequence
  ARTIFICIAL SEQUENCE
GYTYSMGAMA

SEQ ID NO: 64 - protein, 10 aa, Artificial sequence
  ARTIFICIAL SEQUENCE
LIATSSGFIS

SEQ ID NO: 65 - protein, 13 aa, Artificial sequence
  ARTIFICIAL SEQUENCE
GTQFSWSPGSYNY

SEQ ID NO: 66 - protein, 7 aa, Artificial sequence
  ARTIFICIAL SEQUENCE
GYTYSMG

SEQ ID NO: 67 - protein, 6 aa, Artificial sequence
  ARTIFICIAL SEQUENCE
ATSSGF

SEQ ID NO: 68 - protein, 13 aa, Artificial sequence
  ARTIFICIAL SEQUENCE
GTQFSWSPGSYNY

SEQ ID NO: 69 - protein, 8 aa, Artificial sequence
  ARTIFICIAL SEQUENCE
GYTYSMGA

SEQ ID NO: 70 - protein, 8 aa, Artificial sequence
  ARTIFICIAL SEQUENCE
IATSSGFI

SEQ ID NO: 71 - protein, 15 aa, Artificial sequence
  ARTIFICIAL SEQUENCE
AAGTQFSWSPGSYNY

SEQ ID NO: 72 - protein, 5 aa, Artificial sequence
  ARTIFICIAL SEQUENCE
NYDMS

SEQ ID NO: 73 - protein, 17 aa, Artificial sequence
  ARTIFICIAL SEQUENCE
GINSGGGHPHYADSVKG

SEQ ID NO: 74 - protein, 12 aa, Artificial sequence
  ARTIFICIAL SEQUENCE
DEGERYGEDFGY

SEQ ID NO: 75 - protein, 10 aa, Artificial sequence
  ARTIFICIAL SEQUENCE
GFTFSNYDMS

SEQ ID NO: 76 - protein, 10 aa, Artificial sequence
  ARTIFICIAL SEQUENCE
GINSGGGHPH

SEQ ID NO: 77 - protein, 12 aa, Artificial sequence
  ARTIFICIAL SEQUENCE
DEGERYGEDFGY

SEQ ID NO: 78 - protein, 7 aa, Artificial sequence
  ARTIFICIAL SEQUENCE
GFTFSNY

SEQ ID NO: 79 - protein, 6 aa, Artificial sequence
  ARTIFICIAL SEQUENCE
NSGGGH

SEQ ID NO: 80 - protein, 12 aa, Artificial sequence
  ARTIFICIAL SEQUENCE
DEGERYGEDFGY

SEQ ID NO: 81 - protein, 8 aa, Artificial sequence
  ARTIFICIAL SEQUENCE
GFTFSNYD

SEQ ID NO: 82 - protein, 8 aa, Artificial sequence
  ARTIFICIAL SEQUENCE
INSGGGHP

SEQ ID NO: 83 - protein, 14 aa, Artificial sequence
  ARTIFICIAL SEQUENCE
ATDEGERYGEDFGY

SEQ ID NO: 84 - protein, 5 aa, Artificial sequence
  ARTIFICIAL SEQUENCE
NYDMS

SEQ ID NO: 85 - protein, 17 aa, Artificial sequence
  ARTIFICIAL SEQUENCE
GINSGGGHPHYADSVKG

SEQ ID NO: 86 - protein, 12 aa, Artificial sequence
  ARTIFICIAL SEQUENCE
DEGERYGEDFGY

SEQ ID NO: 87 - protein, 10 aa, Artificial sequence
  ARTIFICIAL SEQUENCE
GFTFSNYDMS

SEQ ID NO: 88 - protein, 10 aa, Artificial sequence
  ARTIFICIAL SEQUENCE
GINSGGGHPH

SEQ ID NO: 89 - protein, 12 aa, Artificial sequence
  ARTIFICIAL SEQUENCE
DEGERYGEDFGY

SEQ ID NO: 90 - protein, 7 aa, Artificial sequence
  ARTIFICIAL SEQUENCE
GFTFSNY

SEQ ID NO: 91 - protein, 6 aa, Artificial sequence
  ARTIFICIAL SEQUENCE
NSGGGH

SEQ ID NO: 92 - protein, 12 aa, Artificial sequence
  ARTIFICIAL SEQUENCE
DEGERYGEDFGY

SEQ ID NO: 93 - protein, 8 aa, Artificial sequence
  ARTIFICIAL SEQUENCE
GFTFSNYD

SEQ ID NO: 94 - protein, 8 aa, Artificial sequence
  ARTIFICIAL SEQUENCE
INSGGGHP

SEQ ID NO: 95 - protein, 14 aa, Artificial sequence
  ARTIFICIAL SEQUENCE
ATDEGERYGEDFGY

SEQ ID NO: 96 - protein, 5 aa, Artificial sequence
  ARTIFICIAL SEQUENCE
IYDMS

SEQ ID NO: 97 - protein, 17 aa, Artificial sequence
  ARTIFICIAL SEQUENCE
AINSGGGSTYYADSVKG

SEQ ID NO: 98 - protein, 11 aa, Artificial sequence
  ARTIFICIAL SEQUENCE
GDGGSWYRDGD

SEQ ID NO: 99 - protein, 10 aa, Artificial sequence
  ARTIFICIAL SEQUENCE
GLRFEIYDMS

SEQ ID NO: 100 - protein, 10 aa, Artificial sequence
  ARTIFICIAL SEQUENCE
AINSGGGSTY

SEQ ID NO: 101 - protein, 11 aa, Artificial sequence
  ARTIFICIAL SEQUENCE
GDGGSWYRDGD

SEQ ID NO: 102 - protein, 7 aa, Artificial sequence
  ARTIFICIAL SEQUENCE
GLRFEIY

SEQ ID NO: 103 - protein, 6 aa, Artificial sequence
  ARTIFICIAL SEQUENCE
NSGGGS

SEQ ID NO: 104 - protein, 11 aa, Artificial sequence
  ARTIFICIAL SEQUENCE
GDGGSWYRDGD

SEQ ID NO: 105 - protein, 8 aa, Artificial sequence
  ARTIFICIAL SEQUENCE
GLRFEIYD

SEQ ID NO: 106 - protein, 8 aa, Artificial sequence
  ARTIFICIAL SEQUENCE
INSGGGST

SEQ ID NO: 107 - protein, 13 aa, Artificial sequence
  ARTIFICIAL SEQUENCE
ATGDGGSWYRDGD

SEQ ID NO: 108 - protein, 5 aa, Artificial sequence
  ARTIFICIAL SEQUENCE
LYDMS

SEQ ID NO: 109 - protein, 18 aa, Artificial sequence
  ARTIFICIAL SEQUENCE
GISGESGGSTYYADSVKG

SEQ ID NO: 110 - protein, 11 aa, Artificial sequence
  ARTIFICIAL SEQUENCE
GDRGTWYREDD

SEQ ID NO: 111 - protein, 10 aa, Artificial sequence
  ARTIFICIAL SEQUENCE
GLTFSLYDMS

SEQ ID NO: 112 - protein, 11 aa, Artificial sequence
  ARTIFICIAL SEQUENCE
GISGESGGSTY

SEQ ID NO: 113 - protein, 11 aa, Artificial sequence
  ARTIFICIAL SEQUENCE
GDRGTWYREDD

SEQ ID NO: 114 - protein, 7 aa, Artificial sequence
  ARTIFICIAL SEQUENCE
GLTFSLY

SEQ ID NO: 115 - protein, 7 aa, Artificial sequence
  ARTIFICIAL SEQUENCE
SGESGGS

SEQ ID NO: 116 - protein, 11 aa, Artificial sequence
  ARTIFICIAL SEQUENCE
GDRGTWYREDD

SEQ ID NO: 117 - protein, 8 aa, Artificial sequence
  ARTIFICIAL SEQUENCE
GLTFSLYD

SEQ ID NO: 118 - protein, 9 aa, Artificial sequence
  ARTIFICIAL SEQUENCE
ISGESGGST

SEQ ID NO: 119 - protein, 13 aa, Artificial sequence
  ARTIFICIAL SEQUENCE
ATGDRGTWYREDD

SEQ ID NO: 120 - protein, 5 aa, Artificial sequence
  ARTIFICIAL SEQUENCE
IYDMS

SEQ ID NO: 121 - protein, 17 aa, Artificial sequence
  ARTIFICIAL SEQUENCE
GINSGGGSTYYADSVKG

SEQ ID NO: 122 - protein, 11 aa, Artificial sequence
  ARTIFICIAL SEQUENCE
GLGGSWFREDD

SEQ ID NO: 123 - protein, 10 aa, Artificial sequence
  ARTIFICIAL SEQUENCE
GLRFSIYDMS

SEQ ID NO: 124 - protein, 10 aa, Artificial sequence
  ARTIFICIAL SEQUENCE
GINSGGGSTY

SEQ ID NO: 125 - protein, 11 aa, Artificial sequence
  ARTIFICIAL SEQUENCE
GLGGSWFREDD

SEQ ID NO: 126 - protein, 7 aa, Artificial sequence
  ARTIFICIAL SEQUENCE
GLRFSIY

SEQ ID NO: 127 - protein, 6 aa, Artificial sequence
  ARTIFICIAL SEQUENCE
NSGGGS

SEQ ID NO: 128 - protein, 11 aa, Artificial sequence
  ARTIFICIAL SEQUENCE
GLGGSWFREDD

SEQ ID NO: 129 - protein, 8 aa, Artificial sequence
  ARTIFICIAL SEQUENCE
GLRFSIYD

SEQ ID NO: 130 - protein, 8 aa, Artificial sequence
  ARTIFICIAL SEQUENCE
INSGGGST

SEQ ID NO: 131 - protein, 13 aa, Artificial sequence
  ARTIFICIAL SEQUENCE
ATGLGGSWFREDD

SEQ ID NO: 132 - protein, 5 aa, Artificial sequence
  ARTIFICIAL SEQUENCE
DSDMG

SEQ ID NO: 133 - protein, 16 aa, Artificial sequence
  ARTIFICIAL SEQUENCE
TISSDGRGFYADSVKG

SEQ ID NO: 134 - protein, 9 aa, Artificial sequence
  ARTIFICIAL SEQUENCE
GWYGSFCSG

SEQ ID NO: 135 - protein, 10 aa, Artificial sequence
  ARTIFICIAL SEQUENCE
GFTFDDSDMG

SEQ ID NO: 136 - protein, 9 aa, Artificial sequence
  ARTIFICIAL SEQUENCE
TISSDGRGF

SEQ ID NO: 137 - protein, 9 aa, Artificial sequence
  ARTIFICIAL SEQUENCE
GWYGSFCSG

SEQ ID NO: 138 - protein, 7 aa, Artificial sequence
  ARTIFICIAL SEQUENCE
GFTFDDS

SEQ ID NO: 139 - protein, 5 aa, Artificial sequence
  ARTIFICIAL SEQUENCE
SSDGR

SEQ ID NO: 140 - protein, 9 aa, Artificial sequence
  ARTIFICIAL SEQUENCE
GWYGSFCSG

SEQ ID NO: 141 - protein, 8 aa, Artificial sequence
  ARTIFICIAL SEQUENCE
GFTFDDSD

SEQ ID NO: 142 - protein, 7 aa, Artificial sequence
  ARTIFICIAL SEQUENCE
ISSDGRG

SEQ ID NO: 143 - protein, 11 aa, Artificial sequence
  ARTIFICIAL SEQUENCE
AAGWYGSFCSG

SEQ ID NO: 144 - protein, 5 aa, Artificial sequence
  ARTIFICIAL SEQUENCE
IYDWS

SEQ ID NO: 145 - protein, 17 aa, Artificial sequence
  ARTIFICIAL SEQUENCE
AINSGGGVTSYADSVKG

SEQ ID NO: 146 - protein, 11 aa, Artificial sequence
  ARTIFICIAL SEQUENCE
GDGGSWYRDGD

SEQ ID NO: 147 - protein, 10 aa, Artificial sequence
  ARTIFICIAL SEQUENCE
GLRFSIYDWS

SEQ ID NO: 148 - protein, 10 aa, Artificial sequence
  ARTIFICIAL SEQUENCE
AINSGGGVTS

SEQ ID NO: 149 - protein, 11 aa, Artificial sequence
  ARTIFICIAL SEQUENCE
GDGGSWYRDGD

SEQ ID NO: 150 - protein, 7 aa, Artificial sequence
  ARTIFICIAL SEQUENCE
GLRFSIY

SEQ ID NO: 151 - protein, 6 aa, Artificial sequence
  ARTIFICIAL SEQUENCE
NSGGGV

SEQ ID NO: 152 - protein, 11 aa, Artificial sequence
  ARTIFICIAL SEQUENCE
GDGGSWYRDGD

SEQ ID NO: 153 - protein, 8 aa, Artificial sequence
  ARTIFICIAL SEQUENCE
GLRFSIYD

SEQ ID NO: 154 - protein, 8 aa, Artificial sequence
  ARTIFICIAL SEQUENCE
GLRFSIYD

SEQ ID NO: 155 - protein, 13 aa, Artificial sequence
  ARTIFICIAL SEQUENCE
ATGDGGSWYRDGD

SEQ ID NO: 156 - protein, 10 aa, Artificial sequence
  ARTIFICIAL SEQUENCE
GLISTRHCMS

SEQ ID NO: 157 - protein, 16 aa, Artificial sequence
  ARTIFICIAL SEQUENCE
VIGSDGSTRYGDFAKG

SEQ ID NO: 158 - protein, 23 aa, Artificial sequence
  ARTIFICIAL SEQUENCE
GPLVSTASRRRTRCPEGPRENIY

SEQ ID NO: 159 - protein, 15 aa, Artificial sequence
  ARTIFICIAL SEQUENCE
GLISTGLISTRHCMS

SEQ ID NO: 160 - protein, 9 aa, Artificial sequence
  ARTIFICIAL SEQUENCE
VIGSDGSTR

SEQ ID NO: 161 - protein, 23 aa, Artificial sequence
  ARTIFICIAL SEQUENCE
GPLVSTASRRRTRCPEGPRENIY

SEQ ID NO: 162 - protein, 12 aa, Artificial sequence
  ARTIFICIAL SEQUENCE
GLISTGLISTRH

SEQ ID NO: 163 - protein, 5 aa, Artificial sequence
  ARTIFICIAL SEQUENCE
GSDGS

SEQ ID NO: 164 - protein, 23 aa, Artificial sequence
  ARTIFICIAL SEQUENCE
GPLVSTASRRRTRCPEGPRENIY

SEQ ID NO: 165 - protein, 13 aa, Artificial sequence
  ARTIFICIAL SEQUENCE
GLISTGLISTRHC

SEQ ID NO: 166 - protein, 7 aa, Artificial sequence
  ARTIFICIAL SEQUENCE
IGSDGST

SEQ ID NO: 167 - protein, 25 aa, Artificial sequence
  ARTIFICIAL SEQUENCE
AAGPLVSTASRRRTRCPEGPRENIY

SEQ ID NO: 168 - protein, 5 aa, Artificial sequence
  ARTIFICIAL SEQUENCE
LYDMS

SEQ ID NO: 169 - protein, 17 aa, Artificial sequence
  ARTIFICIAL SEQUENCE
AITNPGGSTYYADSVKD

SEQ ID NO: 170 - protein, 11 aa, Artificial sequence
  ARTIFICIAL SEQUENCE
GRRATFQREKD

SEQ ID NO: 171 - protein, 10 aa, Artificial sequence
  ARTIFICIAL SEQUENCE
GFTFSLYDMS

SEQ ID NO: 172 - protein, 10 aa, Artificial sequence
  ARTIFICIAL SEQUENCE
AITNPGGSTY

SEQ ID NO: 173 - protein, 11 aa, Artificial sequence
  ARTIFICIAL SEQUENCE
GRRATFQREKD

SEQ ID NO: 174 - protein, 7 aa, Artificial sequence
  ARTIFICIAL SEQUENCE
GFTFSLY

SEQ ID NO: 175 - protein, 6 aa, Artificial sequence
  ARTIFICIAL SEQUENCE
TNPGGS

SEQ ID NO: 176 - protein, 11 aa, Artificial sequence
  ARTIFICIAL SEQUENCE
GRRATFQREKD

SEQ ID NO: 177 - protein, 8 aa, Artificial sequence
  ARTIFICIAL SEQUENCE
GFTFSLYD

SEQ ID NO: 178 - protein, 8 aa, Artificial sequence
  ARTIFICIAL SEQUENCE
ITNPGGST

SEQ ID NO: 179 - protein, 13 aa, Artificial sequence
  ARTIFICIAL SEQUENCE
AIGRRATFQREKD

SEQ ID NO: 180 - protein, 5 aa, Artificial sequence
  ARTIFICIAL SEQUENCE
NYCMA

SEQ ID NO: 181 - protein, 16 aa, Artificial sequence
  ARTIFICIAL SEQUENCE
AIYSDGSTSYADSVKG

SEQ ID NO: 182 - protein, 21 aa, Artificial sequence
  ARTIFICIAL SEQUENCE
TAYEGSWTGKQPLCLLYEYTY

SEQ ID NO: 183 - protein, 11 aa, Artificial sequence
  ARTIFICIAL SEQUENCE
GHTYSSNYCMA

SEQ ID NO: 184 - protein, 9 aa, Artificial sequence
  ARTIFICIAL SEQUENCE
AIYSDGSTS

SEQ ID NO: 185 - protein, 21 aa, Artificial sequence
  ARTIFICIAL SEQUENCE
TAYEGSWTGKQPLCLLYEYTY

SEQ ID NO: 186 - protein, 8 aa, Artificial sequence
  ARTIFICIAL SEQUENCE
GHTYSSNY

SEQ ID NO: 187 - protein, 6 aa, Artificial sequence
  ARTIFICIAL SEQUENCE
YSDGST

SEQ ID NO: 188 - protein, 21 aa, Artificial sequence
  ARTIFICIAL SEQUENCE
TAYEGSWTGKQPLCLLYEYTY

SEQ ID NO: 189 - protein, 9 aa, Artificial sequence
  ARTIFICIAL SEQUENCE
GHTYSSNYC

SEQ ID NO: 190 - protein, 7 aa, Artificial sequence
  ARTIFICIAL SEQUENCE
IYSDGST

SEQ ID NO: 191 - protein, 23 aa, Artificial sequence
  ARTIFICIAL SEQUENCE
AATAYEGSWTGKQPLCLLYEYTY

SEQ ID NO: 192 - protein, 5 aa, Artificial sequence
  ARTIFICIAL SEQUENCE
LYDMS

SEQ ID NO: 193 - protein, 17 aa, Artificial sequence
  ARTIFICIAL SEQUENCE
GIGGDGGSTYYADSVKG

SEQ ID NO: 194 - protein, 10 aa, Artificial sequence
  ARTIFICIAL SEQUENCE
GRPPYTDYDS

SEQ ID NO: 195 - protein, 10 aa, Artificial sequence
  ARTIFICIAL SEQUENCE
GFTFSLYDMS

SEQ ID NO: 196 - protein, 10 aa, Artificial sequence
  ARTIFICIAL SEQUENCE
GIGGDGGSTY

SEQ ID NO: 197 - protein, 10 aa, Artificial sequence
  ARTIFICIAL SEQUENCE
GRPPYTDYDS

SEQ ID NO: 198 - protein, 7 aa, Artificial sequence
  ARTIFICIAL SEQUENCE
GFTFSLY

SEQ ID NO: 199 - protein, 6 aa, Artificial sequence
  ARTIFICIAL SEQUENCE
GGDGGS

SEQ ID NO: 200 - protein, 10 aa, Artificial sequence
  ARTIFICIAL SEQUENCE
GRPPYTDYDS

SEQ ID NO: 201 - protein, 8 aa, Artificial sequence
  ARTIFICIAL SEQUENCE
GFTFSLYD

SEQ ID NO: 202 - protein, 8 aa, Artificial sequence
  ARTIFICIAL SEQUENCE
IGGDGGST

SEQ ID NO: 203 - protein, 12 aa, Artificial sequence
  ARTIFICIAL SEQUENCE
ALGRPPYTDYDS

SEQ ID NO: 204 - protein, 5 aa, Artificial sequence
  ARTIFICIAL SEQUENCE
SNFMG

SEQ ID NO: 205 - protein, 17 aa, Artificial sequence
  ARTIFICIAL SEQUENCE
AIYTGGASTFYADSVKG

SEQ ID NO: 206 - protein, 15 aa, Artificial sequence
  ARTIFICIAL SEQUENCE
APRWIAPLRADRYEY

SEQ ID NO: 207 - protein, 10 aa, Artificial sequence
  ARTIFICIAL SEQUENCE
GFTASSNFMG

SEQ ID NO: 208 - protein, 10 aa, Artificial sequence
  ARTIFICIAL SEQUENCE
AIYTGGASTF

SEQ ID NO: 209 - protein, 15 aa, Artificial sequence
  ARTIFICIAL SEQUENCE
APRWIAPLRADRYEY

SEQ ID NO: 210 - protein, 7 aa, Artificial sequence
  ARTIFICIAL SEQUENCE
GFTASSN

SEQ ID NO: 211 - protein, 6 aa, Artificial sequence
  ARTIFICIAL SEQUENCE
YTGGAS

SEQ ID NO: 212 - protein, 15 aa, Artificial sequence
  ARTIFICIAL SEQUENCE
APRWIAPLRADRYEY

SEQ ID NO: 213 - protein, 8 aa, Artificial sequence
  ARTIFICIAL SEQUENCE
GFTASSNF

SEQ ID NO: 214 - protein, 8 aa, Artificial sequence
  ARTIFICIAL SEQUENCE
IYTGGAST

SEQ ID NO: 215 - protein, 17 aa, Artificial sequence
  ARTIFICIAL SEQUENCE
AAAPRWIAPLRADRYEY

SEQ ID NO: 216 - protein, 5 aa, Artificial sequence
  ARTIFICIAL SEQUENCE
DSDMA

SEQ ID NO: 217 - protein, 16 aa, Artificial sequence
  ARTIFICIAL SEQUENCE
TITSDGGTYYADSVKG

SEQ ID NO: 218 - protein, 18 aa, Artificial sequence
  ARTIFICIAL SEQUENCE
DQWGSAEGDCTSSYPGGY

SEQ ID NO: 219 - protein, 10 aa, Artificial sequence
  ARTIFICIAL SEQUENCE
EFTFDDSDMA

SEQ ID NO: 220 - protein, 9 aa, Artificial sequence
  ARTIFICIAL SEQUENCE
TITSDGGTY

SEQ ID NO: 221 - protein, 18 aa, Artificial sequence
  ARTIFICIAL SEQUENCE
DQWGSAEGDCTSSYPGGY

SEQ ID NO: 222 - protein, 7 aa, Artificial sequence
  ARTIFICIAL SEQUENCE
EFTFDDS

SEQ ID NO: 223 - protein, 5 aa, Artificial sequence
  ARTIFICIAL SEQUENCE
TSDGG

SEQ ID NO: 224 - protein, 18 aa, Artificial sequence
  ARTIFICIAL SEQUENCE
DQWGSAEGDCTSSYPGGY

SEQ ID NO: 225 - protein, 8 aa, Artificial sequence
  ARTIFICIAL SEQUENCE
EFTFDDSD

SEQ ID NO: 226 - protein, 7 aa, Artificial sequence
  ARTIFICIAL SEQUENCE
ITSDGGT

SEQ ID NO: 227 - protein, 20 aa, Artificial sequence
  ARTIFICIAL SEQUENCE
AADQWGSAEGDCTSSYPGGY

SEQ ID NO: 228 - protein, 5 aa, Artificial sequence
  ARTIFICIAL SEQUENCE
LYDMS

SEQ ID NO: 229 - protein, 17 aa, Artificial sequence
  ARTIFICIAL SEQUENCE
AIDSGDGRTYYADSVKG

SEQ ID NO: 230 - protein, 11 aa, Artificial sequence
  ARTIFICIAL SEQUENCE
GGRGSWFRESD

SEQ ID NO: 231 - protein, 10 aa, Artificial sequence
  ARTIFICIAL SEQUENCE
GFTFSLYDMS

SEQ ID NO: 232 - protein, 10 aa, Artificial sequence
  ARTIFICIAL SEQUENCE
AIDSGDGRTY

SEQ ID NO: 233 - protein, 11 aa, Artificial sequence
  ARTIFICIAL SEQUENCE
GGRGSWFRESD

SEQ ID NO: 234 - protein, 7 aa, Artificial sequence
  ARTIFICIAL SEQUENCE
GFTFSLY

SEQ ID NO: 235 - protein, 6 aa, Artificial sequence
  ARTIFICIAL SEQUENCE
DSGDGR

SEQ ID NO: 236 - protein, 11 aa, Artificial sequence
  ARTIFICIAL SEQUENCE
GGRGSWFRESD

SEQ ID NO: 237 - protein, 8 aa, Artificial sequence
  ARTIFICIAL SEQUENCE
GFTFSLYD

SEQ ID NO: 238 - protein, 8 aa, Artificial sequence
  ARTIFICIAL SEQUENCE
IDSGDGRT

SEQ ID NO: 239 - protein, 13 aa, Artificial sequence
  ARTIFICIAL SEQUENCE
ANGGRGSWFRESD

SEQ ID NO: 240 - protein, 5 aa, Artificial sequence
  ARTIFICIAL SEQUENCE
YYDMS

SEQ ID NO: 241 - protein, 16 aa, Artificial sequence
  ARTIFICIAL SEQUENCE
AIDARSITDYADAVKG

SEQ ID NO: 242 - protein, 11 aa, Artificial sequence
  ARTIFICIAL SEQUENCE
GGRIGWFREDD

SEQ ID NO: 243 - protein, 10 aa, Artificial sequence
  ARTIFICIAL SEQUENCE
GFTFEYYDMS

SEQ ID NO: 244 - protein, 9 aa, Artificial sequence
  ARTIFICIAL SEQUENCE
AIDARSITD

SEQ ID NO: 245 - protein, 11 aa, Artificial sequence
  ARTIFICIAL SEQUENCE
GGRIGWFREDD

SEQ ID NO: 246 - protein, 7 aa, Artificial sequence
  ARTIFICIAL SEQUENCE
GFTFEYY

SEQ ID NO: 247 - protein, 5 aa, Artificial sequence
  ARTIFICIAL SEQUENCE
DARSI

SEQ ID NO: 248 - protein, 11 aa, Artificial sequence
  ARTIFICIAL SEQUENCE
GGRIGWFREDD

SEQ ID NO: 249 - protein, 8 aa, Artificial sequence
  ARTIFICIAL SEQUENCE
GFTFEYYD

SEQ ID NO: 250 - protein, 7 aa, Artificial sequence
  ARTIFICIAL SEQUENCE
IDARSIT

SEQ ID NO: 251 - protein, 13 aa, Artificial sequence
  ARTIFICIAL SEQUENCE
ANGGRIGWFREDD

SEQ ID NO: 252 - protein, 5 aa, Artificial sequence
  ARTIFICIAL SEQUENCE
NNFVG

SEQ ID NO: 253 - protein, 17 aa, Artificial sequence
  ARTIFICIAL SEQUENCE
AIYSLGGSTYYADSVKG

SEQ ID NO: 254 - protein, 15 aa, Artificial sequence
  ARTIFICIAL SEQUENCE
AITWVPPLSHRRYTY

SEQ ID NO: 255 - protein, 10 aa, Artificial sequence
  ARTIFICIAL SEQUENCE
GYTFNNNFVG

SEQ ID NO: 256 - protein, 10 aa, Artificial sequence
  ARTIFICIAL SEQUENCE
AIYSLGGSTY

SEQ ID NO: 257 - protein, 15 aa, Artificial sequence
  ARTIFICIAL SEQUENCE
AITWVPPLSHRRYTY

SEQ ID NO: 258 - protein, 7 aa, Artificial sequence
  ARTIFICIAL SEQUENCE
GYTFNNN

SEQ ID NO: 259 - protein, 6 aa, Artificial sequence
  ARTIFICIAL SEQUENCE
YSLGGS

SEQ ID NO: 260 - protein, 15 aa, Artificial sequence
  ARTIFICIAL SEQUENCE
AITWVPPLSHRRYTY

SEQ ID NO: 261 - protein, 8 aa, Artificial sequence
  ARTIFICIAL SEQUENCE
GYTFNNNF

SEQ ID NO: 262 - protein, 8 aa, Artificial sequence
  ARTIFICIAL SEQUENCE
IYSLGGST

SEQ ID NO: 263 - protein, 17 aa, Artificial sequence
  ARTIFICIAL SEQUENCE
AGAITWVPPLSHRRYTY

SEQ ID NO: 264 - protein, 5 aa, Artificial sequence
  ARTIFICIAL SEQUENCE
DSDMG

SEQ ID NO: 265 - protein, 16 aa, Artificial sequence
  ARTIFICIAL SEQUENCE
HITNDGTTYYADSVKG

SEQ ID NO: 266 - protein, 16 aa, Artificial sequence
  ARTIFICIAL SEQUENCE
DAWGGGRSTCVNPIGY

SEQ ID NO: 267 - protein, 10 aa, Artificial sequence
  ARTIFICIAL SEQUENCE
GFTFDDSDMG

SEQ ID NO: 268 - protein, 9 aa, Artificial sequence
  ARTIFICIAL SEQUENCE
HITNDGTTY

SEQ ID NO: 269 - protein, 16 aa, Artificial sequence
  ARTIFICIAL SEQUENCE
DAWGGGRSTCVNPIGY

SEQ ID NO: 270 - protein, 7 aa, Artificial sequence
  ARTIFICIAL SEQUENCE
GFTFDDS

SEQ ID NO: 271 - protein, 5 aa, Artificial sequence
  ARTIFICIAL SEQUENCE
TNDGT

SEQ ID NO: 272 - protein, 16 aa, Artificial sequence
  ARTIFICIAL SEQUENCE
DAWGGGRSTCVNPIGY

SEQ ID NO: 273 - protein, 8 aa, Artificial sequence
  ARTIFICIAL SEQUENCE
GFTFDDSD

SEQ ID NO: 274 - protein, 7 aa, Artificial sequence
  ARTIFICIAL SEQUENCE
ITNDGTT

SEQ ID NO: 275 - protein, 18 aa, Artificial sequence
  ARTIFICIAL SEQUENCE
AADAWGGGRSTCVNPIGY

SEQ ID NO: 276 - protein, 5 aa, Artificial sequence
  ARTIFICIAL SEQUENCE
RNIMS

SEQ ID NO: 277 - protein, 15 aa, Artificial sequence
  ARTIFICIAL SEQUENCE
AIDSDGVDYADSVKG

SEQ ID NO: 278 - protein, 13 aa, Artificial sequence
  ARTIFICIAL SEQUENCE
VDFGTTSQCRGNY

SEQ ID NO: 279 - protein, 10 aa, Artificial sequence
  ARTIFICIAL SEQUENCE
GFTGCRNIMS

SEQ ID NO: 280 - protein, 8 aa, Artificial sequence
  ARTIFICIAL SEQUENCE
AIDSDGVD

SEQ ID NO: 281 - protein, 13 aa, Artificial sequence
  ARTIFICIAL SEQUENCE
VDFGTTSQCRGNY

SEQ ID NO: 282 - protein, 7 aa, Artificial sequence
  ARTIFICIAL SEQUENCE
GFTGCRN

SEQ ID NO: 283 - protein, 4 aa, Artificial sequence
  ARTIFICIAL SEQUENCE
DSDG

SEQ ID NO: 284 - protein, 13 aa, Artificial sequence
  ARTIFICIAL SEQUENCE
VDFGTTSQCRGNY

SEQ ID NO: 285 - protein, 8 aa, Artificial sequence
  ARTIFICIAL SEQUENCE
GFTGCRNI

SEQ ID NO: 286 - protein, 6 aa, Artificial sequence
  ARTIFICIAL SEQUENCE
IDSDGV

SEQ ID NO: 287 - protein, 15 aa, Artificial sequence
  ARTIFICIAL SEQUENCE
RRVDFGTTSQCRGNY

SEQ ID NO: 288 - protein, 5 aa, Artificial sequence
  ARTIFICIAL SEQUENCE
NNFVG

SEQ ID NO: 289 - protein, 17 aa, Artificial sequence
  ARTIFICIAL SEQUENCE
TIYTLGSSTYYADSVKG

SEQ ID NO: 290 - protein, 15 aa, Artificial sequence
  ARTIFICIAL SEQUENCE
ARGWVSPLDPARFVY

SEQ ID NO: 291 - protein, 10 aa, Artificial sequence
  ARTIFICIAL SEQUENCE
GYTFSNNFVG

SEQ ID NO: 292 - protein, 10 aa, Artificial sequence
  ARTIFICIAL SEQUENCE
TIYTLGSSTY

SEQ ID NO: 293 - protein, 15 aa, Artificial sequence
  ARTIFICIAL SEQUENCE
ARGWVSPLDPARFVY

SEQ ID NO: 294 - protein, 7 aa, Artificial sequence
  ARTIFICIAL SEQUENCE
GYTFSNN

SEQ ID NO: 295 - protein, 6 aa, Artificial sequence
  ARTIFICIAL SEQUENCE
YTLGSS

SEQ ID NO: 296 - protein, 15 aa, Artificial sequence
  ARTIFICIAL SEQUENCE
ARGWVSPLDPARFVY

SEQ ID NO: 297 - protein, 8 aa, Artificial sequence
  ARTIFICIAL SEQUENCE
GYTFSNNF

SEQ ID NO: 298 - protein, 8 aa, Artificial sequence
  ARTIFICIAL SEQUENCE
IYTLGSST

SEQ ID NO: 299 - protein, 17 aa, Artificial sequence
  ARTIFICIAL SEQUENCE
AAARGWVSPLDPARFVY

SEQ ID NO: 300 - protein, 123 aa, Artificial sequence
  ARTIFICIAL SEQUENCE
QVQLVESGGGSVQAGGSLRLSCAASGYTYSFNSMGWFRQAPGKEREGVAVIYLGSTHYADSVKGRFTISQDNSKNTVYLQMNSLRAEDTAVYYCAADLLEYDGTWFGSTYNYWGQGTLVTVSS

SEQ ID NO: 301 - protein, 123 aa, Artificial sequence
  ARTIFICIAL SEQUENCE
QVQLVESGGGLVQPGGSLRLSCAASGYTYSFNSMGWFRQAPGKGLEGVSVIYLGSTHYADSVKGRFTISRDNSKNTLYLQMNSLRAEDTAVYYCAADLLEYDGTWFGSTYNYWGQGTLVTVSS

SEQ ID NO: 302 - protein, 123 aa, Artificial sequence
  ARTIFICIAL SEQUENCE
QVQLVESGGGLVQPGGSLRLSCAASGYTYSFNSMGWFRQAPGKEREGVAVIYLGSTHYADSVKGRFTISQDNSKNTVYLQMNSLRAEDTAVYYCAADLLEYDGTWFGSTYNYWGQGTLVTVSS

SEQ ID NO: 303 - protein, 123 aa, Artificial sequence
  ARTIFICIAL SEQUENCE
QVQLVESGGGSVQAGGSLRLSCAASGYTYSFNSMGWFRQAPGKGLEGVSVIYLGSTHYADSVKGRFTISQDNSKNTVYLQMNSLRAEDTAVYYCAADLLEYDGTWFGSTYNYWGQGTLVTVSS

SEQ ID NO: 304 - protein, 123 aa, Artificial sequence
  ARTIFICIAL SEQUENCE
QVQLVESGGGSVQAGGSLRLSCAASGYTYSFNSMGWFRQAPGKGLEGVSVIYLGSTHYADSVKGRFTISQDNSKNTLYLQMNSLKPEDTAVYYCAADLLEYDGTWFGSTYNYWGQGTLVTVSS

SEQ ID NO: 305 - protein, 123 aa, Artificial sequence
  ARTIFICIAL SEQUENCE
QVQLVESGGGLVQPGGSLRLSCAASGYTYSFNSMGWFRQAPGKGLEGVSVIYLGSTHYADSVKGRFTISQDNSKNTLYLQMNSLKPEDTAVYYCAADLLEYDGTWFGSTYNYWGQGTLVTVSS

SEQ ID NO: 306 - protein, 122 aa, Artificial sequence
  ARTIFICIAL SEQUENCE
QVQLVESGGGSVQAGGSLRLSCAASGYTYSMGAMAWFRQAPGKEREGVALIATSSGFISYTDSVKGRFTISQDNSKNTVYLQMNSLRAEDTAVYYCAAGTQFSWSPGSYNYWGQGTLVTVSS

SEQ ID NO: 307 - protein, 122 aa, Artificial sequence
  ARTIFICIAL SEQUENCE
QVQLVESGGGLVQPGGSLRLSCAASGYTYSMGAMAWFRQAPGKGLEGVSLIATSSGFISYTDSVKGRFTISRDNSKNTLYLQMNSLRAEDTAVYYCAAGTQFSWSPGSYNYWGQGTLVTVSS

SEQ ID NO: 308 - protein, 122 aa, Artificial sequence
  ARTIFICIAL SEQUENCE
QVQLVESGGGLVQPGGSLRLSCAASGYTYSMGAMAWFRQAPGKEREGVALIATSSGFISYTDSVKGRFTISQDNSKNTVYLQMNSLRAEDTAVYYCAAGTQFSWSPGSYNYWGQGTLVTVSS

SEQ ID NO: 309 - protein, 122 aa, Artificial sequence
  ARTIFICIAL SEQUENCE
QVQLVESGGGSVQAGGSLRLSCAASGYTYSMGAMAWFRQAPGKGLEGVSLIATSSGFISYTDSVKGRFTISQDNSKNTVYLQMNSLRAEDTAVYYCAAGTQFSWSPGSYNYWGQGTLVTVSS

SEQ ID NO: 310 - protein, 122 aa, Artificial sequence
  ARTIFICIAL SEQUENCE
QVQLVESGGGSVQAGGSLRLSCAASGYTYSMGAMAWFRQAPGKGLEGVSLIATSSGFISYTDSVKGRFTISQDNSKNTLYLQMNSLKPEDTAVYYCAAGTQFSWSPGSYNYWGQGTLVTVSS

SEQ ID NO: 311 - protein, 122 aa, Artificial sequence
  ARTIFICIAL SEQUENCE
QVQLVESGGGLVQPGGSLRLSCAASGYTYSMGAMAWFRQAPGKGLEGVSLIATSSGFISYTDSVKGRFTISQDNSKNTLYLQMNSLKPEDTAVYYCAAGTQFSWSPGSYNYWGQGTLVTVSS

SEQ ID NO: 312 - protein, 117 aa, Artificial sequence
  ARTIFICIAL SEQUENCE
QVQLVESGGGSVQAGGSLRLSCTASGFTFDDSDMGWYRQAPGNECELVSTISSDGRGFYADSVKGRFTISQDNSKNTVYLQMNSLRAEDTAVYYCAAGWYGSFCSGLGQGTLVTVSS

SEQ ID NO: 313 - protein, 117 aa, Artificial sequence
  ARTIFICIAL SEQUENCE
QVQLVESGGGLVQPGGSLRLSCAASGFTFDDSDMGWYRQAPGNECELVSTISSDGRGFYADSVKGRFTISRDNSKNTLYLQMNSLRAEDTAVYYCAAGWYGSFCSGLGQGTLVTVSS

SEQ ID NO: 314 - protein, 117 aa, Artificial sequence
  ARTIFICIAL SEQUENCE
QVQLVESGGGLVQPGGSLRLSCTASGFTFDDSDMGWYRQAPGNECELVSTISSDGRGFYADSVKGRFTISRDNSKNTVYLQMNSLRAEDTAVYYCAAGWYGSFCSGLGQGTLVTVSS

SEQ ID NO: 315 - protein, 117 aa, Artificial sequence; identical to SEQ ID NO: 312
  ARTIFICIAL SEQUENCE

SEQ ID NO: 316 - protein, 117 aa, Artificial sequence
  ARTIFICIAL SEQUENCE
QVQLVESGGGSVQAGGSLRLSCTASGFTFDDSDMGWYRQAPGNECELVSTISSDGRGFYADSVKGRFTISQDNSKNTLYLQMNSLKPEDTAVYYCAAGWYGSFCSGLGQGTLVTVSS

SEQ ID NO: 317 - protein, 117 aa, Artificial sequence
  ARTIFICIAL SEQUENCE
QVQLVESGGGLVQPGGSLRLSCTASGFTFDDSDMGWYRQAPGNECELVSTISSDGRGFYADSVKGRFTISRDNSKNTLYLQMNSLKPEDTAVYYCAAGWYGSFCSGLGQGTLVTVSS

SEQ ID NO: 318 - protein, 130 aa, Artificial sequence
  ARTIFICIAL SEQUENCE
QVQLVESGGGSVQAGGSLRLSCAASGHTYSSNYCMAWFRQAPGKEREGVAAIYSDGSTSYADSVKGRFTISKDNSKNTLYLQMNSLRAEDTAVYYCAATAYEGSWTGKQPLCLLYEYTYWGQGTLVTVSS

SEQ ID NO: 319 - protein, 130 aa, Artificial sequence
  ARTIFICIAL SEQUENCE
QVQLVESGGGLVQPGGSLRLSCAASGHTYSSNYCMAWFRQAPGKEREGVAAIYSDGSTSYADSVKGRFTISRDNSKNTLYLQMNSLRAEDTAVYYCAATAYEGSWTGKQPLCLLYEYTYWGQGTLVTVSS

SEQ ID NO: 320 - protein, 130 aa, Artificial sequence
  ARTIFICIAL SEQUENCE
QVQLVESGGGLVQPGGSLRLSCAASGHTYSSNYCMAWFRQAPGKEREGVAAIYSDGSTSYADSVKGRFTISKDNSKNTLYLQMNSLRAEDTAVYYCAATAYEGSWTGKQPLCLLYEYTYWGQGTLVTVSS

SEQ ID NO: 321 - protein, 130 aa, Artificial sequence
  ARTIFICIAL SEQUENCE
QVQLVESGGGSVQAGGSLRLSCAASGHTYSSNYCMAWFRQAPGKGLEGVSAIYSDGSTSYADSVKGRFTISKDNSKNTLYLQMNSLRAEDTAVYYCAATAYEGSWTGKQPLCLLYEYTYWGQGTLVTVSS

SEQ ID NO: 322 - protein, 130 aa, Artificial sequence
  ARTIFICIAL SEQUENCE
QVQLVESGGGSVQAGGSLRLSCAASGHTYSSNYCMAWFRQAPGKGLEGVSAIYSDGSTSYADSVKGRFTISKDNSKNTLYLQMNSLKPEDTAVYYCAATAYEGSWTGKQPLCLLYEYTYWGQGTLVTVSS

SEQ ID NO: 323 - protein, 130 aa, Artificial sequence
  ARTIFICIAL SEQUENCE
QVQLVESGGGLVQPGGSLRLSCAASGHTYSSNYCMAWFRQAPGKGLEGVSAIYSDGSTSYADSVKGRFTISKDNSKNTLYLQMNSLKPEDTAVYYCAATAYEGSWTGKQPLCLLYEYTYWGQGTLVTVSS

SEQ ID NO: 324 - protein, 126 aa, Artificial sequence
  ARTIFICIAL SEQUENCE
QVQLVESGGGSVQAGGSLRLSCTASEFTFDDSDMAWYRQAPGNECELVSTITSDGGTYYADSVKGRFTISQDNSKNTMYLQMNSLRAEDTAVYYCAADQWGSAEGDCTSSYPGGYWGQGTLVTVSS

SEQ ID NO: 325 - protein, 126 aa, Artificial sequence
  ARTIFICIAL SEQUENCE
QVQLVESGGGLVQPGGSLRLSCAASEFTFDDSDMAWYRQAPGNECELVSTITSDGGTYYADSVKGRFTISRDNSKNTLYLQMNSLRAEDTAVYYCAADQWGSAEGDCTSSYPGGYWGQGTLVTVSS

SEQ ID NO: 326 - protein, 126 aa, Artificial sequence
  ARTIFICIAL SEQUENCE
QVQLVESGGGLVQPGGSLRLSCTASEFTFDDSDMAWYRQAPGNECELVSTITSDGGTYYADSVKGRFTISQDNSKNTMYLQMNSLRAEDTAVYYCAADQWGSAEGDCTSSYPGGYWGQGTLVTVSS

SEQ ID NO: 327 - protein, 126 aa, Artificial sequence
  ARTIFICIAL SEQUENCE
QVQLVESGGGSVQAGGSLRLSCTASEFTFDDSDMAWYRQAPGNECELVSTITSDGGTYYADSVKGRFTISRDNSKNTMYLQMNSLRAEDTAVYYCAADQWGSAEGDCTSSYPGGYWGQGTLVTVSS

SEQ ID NO: 328 - protein, 126 aa, Artificial sequence
  ARTIFICIAL SEQUENCE
QVQLVESGGGSVQAGGSLRLSCTASEFTFDDSDMAWYRQAPGNECELVSTITSDGGTYYADSVKGRFTISRDNSKNTLYLQMNSLKPEDTAVYYCAADQWGSAEGDCTSSYPGGYWGQGTLVTVSS

SEQ ID NO: 329 - protein, 126 aa, Artificial sequence
  ARTIFICIAL SEQUENCE
QVQLVESGGGLVQPGGSLRLSCTASEFTFDDSDMAWYRQAPGNECELVSTITSDGGTYYADSVKGRFTISRDNSKNTLYLQMNSLKPEDTAVYYCAADQWGSAEGDCTSSYPGGYWGQGTLVTVSS

SEQ ID NO: 330 - protein, 124 aa, Artificial sequence
  ARTIFICIAL SEQUENCE
QVQLVESGGGSVQAGGSLRLSCAASGYTFNNNFVGWFRQAPGKEREGVAAIYSLGGSTYYADSVKGRFTISQDNSKNTVYLQMNSLRAEDTAVYYCAGAITWVPPLSHRRYTYWGQGTLVTVSS

SEQ ID NO: 331 - protein, 124 aa, Artificial sequence
  ARTIFICIAL SEQUENCE
QVQLVESGGGLVQPGGSLRLSCAASGYTFNNNFVGWFRQAPGKGLEGVSAIYSLGGSTYYADSVKGRFTISRDNSKNTLYLQMNSLRAEDTAVYYCAAAITWVPPLSHRRYTYWGQGTLVTVSS

SEQ ID NO: 332 - protein, 124 aa, Artificial sequence
  ARTIFICIAL SEQUENCE
QVQLVESGGGLVQPGGSLRLSCAASGYTFNNNFVGWFRQAPGKEREGVAAIYSLGGSTYYADSVKGRFTISQDNSKNTVYLQMNSLRAEDTAVYYCAGAITWVPPLSHRRYTYWGQGTLVTVSS

SEQ ID NO: 333 - protein, 124 aa, Artificial sequence
  ARTIFICIAL SEQUENCE
QVQLVESGGGSVQAGGSLRLSCAASGYTFNNNFVGWFRQAPGKGLEGVSAIYSLGGSTYYADSVKGRFTISQDNSKNTVYLQMNSLRAEDTAVYYCAGAITWVPPLSHRRYTYWGQGTLVTVSS

SEQ ID NO: 334 - protein, 124 aa, Artificial sequence
  ARTIFICIAL SEQUENCE
QVQLVESGGGSVQAGGSLRLSCAASGYTFNNNFVGWFRQAPGKGLEGVSAIYSLGGSTYYADSVKGRFTISQDNSKNTLYLQMNSLKPEDTAVYYCAGAITWVPPLSHRRYTYWGQGTLVTVSS

SEQ ID NO: 335 - protein, 124 aa, Artificial sequence
  ARTIFICIAL SEQUENCE
QVQLVESGGGSVQAGGSLRLSCAASGYTFNNNFVGWFRQAPGKGLEGVSAIYSLGGSTYYADSVKGRFTISRDNSKNTLYLQMNSLKPEDTAVYYCAGAITWVPPLSHRRYTYWGQGTLVTVSS

SEQ ID NO: 336 - protein, 232 aa, Artificial sequence
  ARTIFICIAL SEQUENCE
EPKSCDKTHTCPPCPAPELLGGPSVFLFPPKPKDTLMISRTPEVTCVVVDVSHEDPEVKFNWYVDGVEVHNAKTKPREEQYNSTYRVVSVLTVLHQDWLNGKEYKCKVSNKALPAPIEKTISKAKGQPREPQVYTLPPSRDELTKNQVSLTCLVKGFYPSDIAVEWESNGQPENNYKTTPPVLDSDGSFFLYSKLTVDKSRWQQGNVFSCSVMHEALHNHYTQKSLSLSPGK

SEQ ID NO: 337 - protein, 91 aa, Artificial sequence
  ARTIFICIAL SEQUENCE
ECVTQLLKDTCFEGGDITTVFTPSAKYCQVVCTYHPRCLLFTFTAESPSEDPTRWFTCVLKDSVTETLPRVNRTAAISGYSFKQCSHQISA

SEQ ID NO: 338 - protein, 95 aa, Artificial sequence
  ARTIFICIAL SEQUENCE
HQISACNKDIYVDLDMKGINYNSSVAKSAQECQERCTDDVHCHFFTYATRQFPSLEHRNICLLKHTQTGTPTRITKLDKVVSGFSLKSCALSNLA

SEQ ID NO: 339 - protein, 96 aa, Artificial sequence
  ARTIFICIAL SEQUENCE
LSNLACIRDIFPNTVFADSNIDSVMAPDAFVCGRICTHHPGCLFFTFFSQEWPKESQRNLCLLKTSESGLPSTRIKKSKALSGFSLQSCRHSIPVF

SEQ ID NO: 340 - protein, 97 aa, Artificial sequence
  ARTIFICIAL SEQUENCE
IPVFCHSSFYHDTDFLGEELDIVAAKSHEACQKLCTNAVRCQFFTYTPAQASCNEGKGKCYLKLSSNGSPTKILHGRGGISGYTLRLCKMDNESTTK

SEQ ID NO: 341 - protein, 181 aa, Artificial sequence
  ARTIFICIAL SEQUENCE
ECVTQLLKDTCFEGGDITTVFTPSAKYCQVVCTYHPRCLLFTFTAESPSEDPTRWFTCVLKDSVTETLPRVNRTAAISGYSFKQCSHQISACNKDIYVDLDMKGINYNSSVAKSAQECQERCTDDVHCHFFTYATRQFPSLEHRNICLLKHTQTGTPTRITKLDKVVSGFSLKSCALSNLA

SEQ ID NO: 342 - protein, 186 aa, Artificial sequence
  ARTIFICIAL SEQUENCE
HQISACNKDIYVDLDMKGINYNSSVAKSAQECQERCTDDVHCHFFTYATRQFPSLEHRNICLLKHTQTGTPTRITKLDKVVSGFSLKSCALSNLACIRDIFPNTVFADSNIDSVMAPDAFVCGRICTHHPGCLFFTFFSQEWPKESQRNLCLLKTSESGLPSTRIKKSKALSGFSLQSCRHSIPVF

SEQ ID NO: 343 - protein, 186 aa, Artificial sequence; identical to SEQ ID NO: 342
  ARTIFICIAL SEQUENCE